European Patent Specification EP 4 426 859 B1, published April 15, 2026. Title: PRIMER SETS AND METHODS AND KITS INCORPORATING THE PRIMER SETS. Applicant: Illumina, Inc. Application US, filed November 1, 2022. The sequence listing filed with the application follows.

SEQUENCE LISTING (12 sequences)

SEQ ID NO: 1 - DNA, 29 bp, synthetic construct
  source 1..29: mol_type = other DNA
  modified_base 23: mod_base = OTHER; note = URACIL
aatgatacggcgaccaccgagatctacac

SEQ ID NO: 2 - DNA, 24 bp, synthetic construct
  source 1..24: mol_type = other DNA
  modified_base 22: mod_base = OTHER; note = 8-oxoguanine
caagcagaagacggcatacganat

SEQ ID NO: 3 - DNA, 24 bp, synthetic construct
  source 1..24: mol_type = other DNA
  modified_base 20: mod_base = OTHER; note = 8-oxoguanine
caagcagaagacggcatacnagat

SEQ ID NO: 4 - DNA, 29 bp, synthetic construct
  source 1..29: mol_type = other DNA
  modified_base 23: mod_base = OTHER; note = allyl-T
aatgatacggcgaccaccgaganctacac

SEQ ID NO: 5 - DNA, 35 bp, synthetic construct
  source 1..35: mol_type = other DNA
gctggcacgtccgaacgcttcgttaatccgttgag

SEQ ID NO: 6 - DNA, 35 bp, synthetic construct
  source 1..35: mol_type = other DNA
ctcaacggattaacgaagcgttcggacgtgccagc

SEQ ID NO: 7 - DNA, 35 bp, synthetic construct
  source 1..35: mol_type = other DNA
cgtcgtctgccatggcgcttcggtggatatgaact

SEQ ID NO: 8 - DNA, 35 bp, synthetic construct
  source 1..35: mol_type = other DNA
agttcatatccaccgaagcgccatggcagacgacg

SEQ ID NO: 9 - DNA, 35 bp, synthetic construct
  source 1..35: mol_type = other DNA
acggccgctaatatcaacgcgtcgaatccgcaact

SEQ ID NO: 10 - DNA, 35 bp
agttgcggattcgacgcgttgatattagcggccgt

SEQ ID NO: 11 - DNA, 34 bp, synthetic construct
  source 1..34: mol_type = other DNA
gccgcgttacgttagccggactattcgatgcagc

SEQ ID NO: 12 - DNA, 34 bp, synthetic construct
  source 1..34: mol_type = other DNA
gctgcatcgaatagtccggctaacgtaacgcggc